European Patent Specification EP 3 390 641 B1, published August 9, 2023. Title: COMPOSITIONS AND METHODS FOR MANIPULATING THE DEVELOPMENT OF PLANTS. Applicant: THE NEW ZEALAND INSTITUTE FOR PLANT AND FOOD RESEARCH LIMITED. The sequence listing filed with the application follows.

SEQUENCE LISTING (29 sequences)

SEQ ID NO: 1 - protein, 708 aa, Malus domestica
  misc_feature (106)..(106): Xaa can be any naturally occurring amino acid
  misc_feature (359)..(359): Xaa can be any naturally occurring amino acid
  misc_feature (403)..(403): Xaa can be any naturally occurring amino acid
  misc_feature (405)..(405): Xaa can be any naturally occurring amino acid
  misc_feature (412)..(412): Xaa can be any naturally occurring amino acid
  misc_feature (469)..(469): Xaa can be any naturally occurring amino acid
  misc_feature (540)..(540): Xaa can be any naturally occurring amino acid
MAGLIDLNSATEDEETPSSGSPSSASSVSDALGSSASVCMELWHACAGPLISLPKKGSVVVYLPQGHLEQVSDFPTSAYDLPPHLFCRVVDVKLHAETGTDDVFAXVSLVPESEEIEHRLREGVTDADAEEDVEAMGTSTTPHMFCKTLTASDTSTHGGFSVPRRAAEDCFPPLDYTQQRPSQELVAKDLHGLEWRFRHIYRGQPRRHLLTTGWSAFVNKKKLVSGDAVLFLRGDDGELRLGIRRAAQFKSSATCPTLCSQQLNYSTITDVVNAIFAKNAFNVYYNPRSSSSEFIIPSHKFLRSLDHCFCAGMRIKMRFETEDAAERRYTGLITGISELDPVRWPGSKWRCLVVRWDDXDTSKHGRVSPWEVERSGSVSSSHTLMTTGLKRSRIGLSATKPEXPXPSMSCNXGIGTSDFGESLRFQKVLQGQEISGFDTPFSGLGGLNSHPSEARRVFHGSGGSGIAAXGNGLRQSLVDSEIASKGIGFGESFRFHKVLQGQEIFPSSPYGRAPASNEAHEYGGPGLYDGFQVPGFRNGXSTMMQSNNTNVHSSAPSVQVSSPSSVLMFQQAMNPVAEFNSVYNGHNQEDHRVNRTPHVLEHDGGRQTSSSFGERNFSREDRGGTHSYNQHGISPHPVISQSTISGSQDSVSPIKGSCRLFGFSLSEDKCVPDQEGNPNVGVQFHSKPPLMTSTVGITCTKVSNLFAA

SEQ ID NO: 2 - protein, 708 aa, Malus domestica
  misc_feature (106)..(106): Xaa can be any naturally occurring amino acid
  misc_feature (359)..(359): Xaa can be any naturally occurring amino acid
  misc_feature (403)..(403): Xaa can be any naturally occurring amino acid
  misc_feature (405)..(405): Xaa can be any naturally occurring amino acid
  misc_feature (412)..(412): Xaa can be any naturally occurring amino acid
  misc_feature (469)..(469): Xaa can be any naturally occurring amino acid
  misc_feature (540)..(540): Xaa can be any naturally occurring amino acid
MAGLIDLNSATEDEETPSSGSPSSASSVSDALGSSASVCMELWHACAGPLISLPKKGSVVVYLPQGHLEQVLDFPTSAYDLPPHLFCRVVDVKLHAETGTDDVFAXVSLVPESEEIEHRLREGVTDADAEEDVEAMGTSTTPHMFCKTLTASDTSTHGGFSVPRRAAEDCFPPLDYTQQRPSQELVAKDLHGLEWRFRHIYRGQPRRHLLTTGWSAFVNKKKLVSGDAVLFLRGDDGELRLGIRRAAQFKSSATCPTLCSQQLNYSTITDVVNAIFAKNAFNVYYNPRSSSSEFIIPSHKFLRSLDHCFCAGMRIKMRFETEDAAERRYTGLITGISELDPVRWPGSKWRCLVVRWDDXDTSKHGRVSPWEVERSGSVSSSHTLMTTGLKRSRIGLSATKPEXPXPSMSCNXGIGTSDFGESLRFQKVLQGQEISGFDTPFSGLGGLNSHPSEARRVFHGSGGSGIAAXGNGLRQSLVDSEIASKGIGFGESFRFHKVLQGQEIFPSSPYGRAPASNEAHEYGGPGLYDGFQVPGFRNGXSTMMQSNNTNVHSSAPSVQVSSPSSVLMFQQAMNPVAEFNSVYNGHNQEDHRVNRTPHVLEHDGGRQTSSSFGERNFSREDRGGTHSYNQHGISPHPVISQSTISGSQDSVSPIKGSCRLFGFSLSEDKCVPDQEGNPNVGVQFHSKPPLMTSTVGITCTKVSNLFAA

SEQ ID NO: 3 - protein, 608 aa, Arabidopsis thaliana
MGGLIDLNVMETEEDETQTQTPSSASGSVSPTSSSSASVSVVSSNSAGGGVCLELWHACAGPLISLPKRGSLVLYFPQGHLEQAPDFSAAIYGLPPHVFCRILDVKLHAETTTDEVYAQVSLLPESEDIERKVREGIIDVDGGEEDYEVLKRSNTPHMFCKTLTASDTSTHGGFSVPRRAAEDCFPPLDYSQPRPSQELLARDLHGLEWRFRHIYRGQPRRHLLTTGWSAFVNKKKLVSGDAVLFLRGDDGKLRLGVRRASQIEGTAALSAQYNQNMNHNNFSEVAHAISTHSVFSISYNPKASWSNFIIPAPKFLKVVDYPFCIGMRFKARVESEDASERRSPGIISGISDLDPIRWPGSKWRCLLVRWDDIVANGHQQRVSPWEIEPSGSISNSGSFVTTGPKRSRIGFSSGKPDIPVSEGIRATDFEESLRFQRVLQGQEIFPGFINTCSDGGAGARRGRFKGTEFGDSYGFHKVLQGQETVPAYSITDHRQQHGLSQRNIWCGPFQNFSTRILPPSVSSSPSSVLLTNSNSPNGRLEDHHGGSGRCRLFGFPLTDETTAVASATAVPCVEGNSMKGASAVQSNHHHSQGRDIYAMRDMLLDIAL

SEQ ID NO: 4 - protein, 730 aa, Phaseolus vulgaris
MVGIIDLNTTEEDEKTTPSSGSFSSPSSSSSTSAALSATNLSSAPVSGSVCLELWHACAGPLISLPKKGSVVVYFPQGHLEQLPDLPLAVYDLPSYIFCRVVDVKLHAETANDEVYAQVSLVPDSEQIEQKLKQGKLEGHCEEEDVEAVVKSTTTHMFCKTLTASDTSTHGGFSVPRRAAEDCFPPLDYSQQRPSQELVAKDLHGFEWKFRHIYRGQPRRHLLTTGWSAFVNKKKLVSGDAVLFLRGDDGELRLGIRRAAQVKCGASFPALCSQQLNQSTLTDVVHAMSMRSLFNICYNPRASSSEFIIPLHKFLKSLDYSFSVGMRFKMRFETEDAAERRYMGLITGISDLDPARWPGSKWRCLVVRWDDMETNRHSRVSPWEIEPSGSVSSCNSFMTPGLKRSRSGFPSSKPEFPVPDGIGASDFGEPSRFQKVLQGQEILNFNTLYDGVDQNRHPSDIRRCFPGSRSSMIATTRNGARDPVVNSDVSYKSIGFSESLRFHKVLQGQEIIPSSPFGRAPASTNEACENGCFGISDGVQMTSSRNGWSSMMQGYNTRIRPPAQVSSPCSVLMFQQASNQVSNPSPRYGFNDLEEQGVNTQSWFHNPETCGEKRMSSSRSEHIFRRNNQWGMDSFSLSHEHSQHGLLQPLVAQPPCKGGQDLVSSCKSSCRLFGFQLTEDRHVANKDDSSIPMASLNAGSFMPHAGEQFHLKPPAITNAVGSSCTKVSVL

SEQ ID NO: 5 - protein, 747 aa, Solanum lycopersicum
MMCGLIDLNTVDNDDAGEETTAPVSLDSPASSSAASGSSDLTSSTTPAVASVCMELWHACAGPLISLPKKGSAVVYLPQGHLEHLSEYPSIACNLPPHVFCRVVDVKLQADAATDEVYAQVSLVPDNQQIEQKWKDGDIDADIEEEEIEGAGKSITPHMFCKTLTASDTSTHGGFSVPRRAAEDCFAPLDYRQQRPSQELVAKDLHGIEWKFRHIYRGQPRRHLLTTGWSAFVNKKKLVSGDAVLFLRTGDGELRLGVRRAAQAKTCSSYLAPCSKPLNVSGIVDAVNVISSRNAFNICYNPRDSSSDFIVPYHKFSKTLAHPFSAGMRFKMRVETEDAAEQRFTGLVVGVSNVDPVRWPGSKWRCLLVRWDDLDVSRHNRVSPWEIEPSGSAPVPSSLVMPSAKRTRVGFPISKADFPIPREGIAVSDFGEPSRFQKVLQGQEILRMHAPYGGLDARSPRPAGTRCFPGFPSSGISRMGNSIRPLFGDTDKSHESIGFSESLRFNKVLQGQEIFTSPPYGRAQAGIQMQEKSRTGIFVGIQVPNHGNRWPAPNQDNNTPCKPINPVSASSPPSALNFQHPSPPASKFQAMFNHKHDLVNQASLDLSENCCRYPYLSSGSHTEDISQKEGTQGISSFGFLKEQKQTGLSYLSPGTQSSFKGNQNLVSTCKTGCRIFGFPLTESKISATRADTPSEAVYSHGLETTFLPSSDGKLQPGPPLMTNVVGTNFTKVNDLYAARDVLLDIAL

SEQ ID NO: 6 - protein, 743 aa, Citrus clemantina
MVGLIDLNTTEDDENPSSGSLSPSSSSASALSASGFALAPASASASGVSLELWHACAGPLISLPKRGSVVVYFPQGHLEHVSDFSAAASAAYDLPPHLFCRVADVKLHAEAASDEVYAQVSLVPDELIEQKVREGKIEEDGDEESVEVVAKSSTPHMFCKTLTASDTSTHGGFSVPRRAAEDCFPPLDYSQQRPSQELVAKDLHGLEWRFRHIYRGQPRRHLLTTGWSAFVNKKKLVSGDAVLFLRGEDGELRLGIRRAPHVKSGATFPSFCSQQSSPNSVTEVVDAIARKRAFSISYNPRASASEFIIPVNKFLKSLGHSFAVGMRFKMRFETEDAAERRYTGVIMGVGDMDPVRWPGSKWRCLLVRWDDVESNRHTRVSPWEIEPSGSVCGSNNLITSGLKRTRIGLPSGKPEFPVPDGIGVTDFGESLRFQKVLQGQEILGFNTLYDGGDCQNLHPSEVRRGIPGSNGSGIAAIGDGSRNLQVKSDISYKGIGIGFGESFRFHKVLQGQEIFPKSPYGRAPTNNEARSIGSLGISDGVPVSGSRNRWSAVVPGYNTHMSPSAPPVQVSSPSSVLMFQLASNPISNYNPPYSLNDQEKEQRVNCQSFFHNSEIYGGKHASSSFLDHSFVGGDQEVMDSIGQSNEHISPPLVGQPTVRGSQDLVSSCKGSCRLFGFSLTEERHVANIEDNAAPVASPLNPRSSFLSHVGQQFHPKPPVMSKATGSNCTNGIMQHCLGNYDIY

SEQ ID NO: 7 - protein, 720 aa, Fragaria vesca
MAGLIDLNSTTEEEEETPSSGSSSNSSGSNGLISGSVCLELWHACAGPLISLPKKGSVVVYLPQGHLEQVSDFPASVYDLPAHLFCRVLDVKLHAESGSDEVYAQVQLVPESEEFEHKLGERETVADGDEDAEGSEKSTTPHMFCKTLTASDTSTHGGFSVPRRAAEDCFPPLDYSQQRPSQELVAKDLHGLEWRFRHIYRGQPRRHLLTTGWSAFVNKKKLVSGDAVLFLRGEDGELRLGVRRAAQVKASATYPTPGSQHLNYNSVTELVDAISTKTAFNAYYNPRASSSEFIIPFRKFLRSLGHSFCAGMRFKMRFETEDAAEQRYTGLVTGISELDPLRWPGSKWKCVAVRWDDIDTSKQHGRVSPWEIEPSGSISNSSGLMASGLKRSRMGLSAEKQEFPVPHGIGASDFGESLRFQKVLQGQEVSGFDTPFGSIGGQNQHPSESRRVFHGSIGSRGNDLRNSFVNSEIASKGFGESFRFQKVLQGQEIFPSTPYGRAPATNEAREYGCPGIFDGFQVPSFRNGWSTMMQGSNTPMHRAAPVQVSSPSSVLMFQQAINAGAEFNSVYNGHNQQEQRIMQRTHSESDGGKQTSASFCERSFTREGHGGMNSFDQHGISHPPLLSQSSLRGSQDMVSSCKSSCRLFGFSLSEETHAPNKVDNSTSVTSALESGASMFPNVEPRFHSKPPSMSAAVGIPCTKEWAFNWRGERMESCLQG

SEQ ID NO: 8 - protein, 722 aa, Prunus persica
MGGLIDLNSATEDEETPSSGSSSTSSASDASASASASVCLELWHACAGPLISLPKKGSVVVYLPQGHLEQVSDFPASAYNLPPHLFCRVVDVKLHAETGTDDVYAQVSLVPESEEIEHKLREGETDAYGEEEDVEAIGKSTTPHMFCKTLTASDTSTHGGFSVPRRAAEDCFPPLDYNQQRPSQELVAKDLHGLEWRFRHIYRGQPRRHLLTTGWSAFVNKKKLVSGDAVLFLRGDDGELRLGIRRAAQVKGSATYPTLCSQQLNYNTITDVVNAISMKNAFNIFYNPRASSSEFIIPSRKFLRSLDHSFSPGMRFKMRFETEDAAERRYTGLITGISELDPVRWPGSKWRCLVVRWDDIDTSKHGRVSPWEIEPSGSVSSSHSLMAAGLKRARSGLSAAKTEFPVPNGIGASDFGESLRFQKVLQGQEILGFDTHFGGLGGQNQHPSEPRRGFHGSSGSGIAAGGNGLRKSLAHSEITSTGIGFGESFRFHKVLQGQEIFPSPPYGRASTNNEAHEYGGPGIYDGFQVPSFRNGWPAMMQSNNAHVRPSASSVQVSSPSSVLMFQQAMNPGPEFNSVYNGHNQEEQRVIKRTPYVSESDGGKQASSSFCERSFSREDHGGMNSYNQHGISNHPVISQSTFSGSQDAVSPYKGSCRLFGFSLSEEKRVPDRESNSTSTASTLNPGVQFHSKPALMTSAVGITCTKEWAFDWRGERMESCLQG

SEQ ID NO: 9 - protein, 704 aa, Pyrus communis
MAGLIDLNSATEDEQTPSSGSPSSASSVSDALGSSASVCMELWHACAGPLISLPKKGSVVVYLPQGHLEQVSDFPTSAYDLPPHLFCRVVDVKLHAETGTDDVFARVSLVPESEEIEHRLREGETDADAEDDVEAMGTSATPHMFCKTLTASDTSTHGGFSVPRRAAEDCFPPLDYTQQRPSQELVAKDLHGLEWRFRHIYRGQPRRHLLTTGWSAFVNKKKLVSGDAVLFLRGDDGELRLGIRRAAQFKSSATCPTLCSQQLNCSAITDVLNAIFAKNAFNVYYNPRSSSSEFIIPSHKFLRSLDHCFSAGMRIKMRFETEDAAERRYIGFITRISELDPVRWPGSKWRCLVVRWDDIDTSKHSRVSPWEVEPSGSVSSSHTLMATGLKRSRIGLSATKPECSVPNGGIGTSDFGESLRFQKVLQGQEISGFDTPFSGLGGLNSLPSEARRVFHGSGGSGIAAGGNGLRQSLVDSEIASKGIGFGESFRFRKVLQGQEILPSSPYGRAPASNEAHEYGGPGIYDGFHVPGFRNGWSTMMQSNNTHVHSSAPSVQVSSPSSVLMFQQAVNPVVEFNSVYNGHNPEDHRVNRTLHVSEHDGGRQTSSSFGELNFSREDRGGTHSYNQHGISPHPGTSQSTISGSQDSISPIKGSCRLFGFSLSEDKCVPDQEGNPNVGVRFHSKPSLMTSTVGITCTKVSNLFAA

SEQ ID NO: 10 - protein, 709 aa, Populus tremula
MVGMIDLNTTEEDETTPSSGSLSSPSSSSAASALSASGSGSGTSPVCLELWHACAGPLISLPKRGSIVVYVPQGHLEQLPDLPLGIYDLPPHVFCRVVDVKLHAEAASDDVYAQVSLVPESEEIEQKLREGVFEGDGEEEDVEATVKTTTPHMFCKTLTASDTSTHGGFSVPRRAAEDCFPPLDYTQQRPSQELVAKDLHGSEWKFRHIYRGQPRRHLLTTGWSAFVNKKKLVSGDAVLFLRGEDGELRLGVRRAAQVKCGPTFPALWNQQLNQSSLADVANAISMRSAFRIYYNPRASSSEFIIPFNKFLKSLDQSFSAGMRVKMRFETEDAAERRYTGLITGISELDPTRWPGSKWKCLLVRWDDTEANRHSRVSPWEVEPSGSVSGSGSGSISSSNNSMAPGLKRSRSGLPSLKAEFPIPDGIGASDFRVSSRFQEVLQGQEIMRSGIRGSIPTSENSFKGIGFNESYRFHKVLQGQEIFPRSPYRRIPNANKARENCGLGLSDGVQRSSSRNGWSTMMQGYNTQMRPPTQVSSPSSVLMFQHASNQVSNPTSIFNSNDHEEQTTNTQSWFYPETHGGKFKLSSHSDPGLRGDSQCSTNPYVLSHEHLQHGISQPVVAQSAFRSSQDMVLCKSSCRLFGFSLTEDRHVVNKEDNIASITSPLNPESSFLPRVGEQLHPKPPAINNAVGSSCTKAIRQHHAENYRIY

SEQ ID NO: 11 - protein, 786 aa, Vitis vinifera
MVAMIDLNTVDDDETPSSGSSSSSSSSASASASTVCGSLLSAASSVCLELWHACAGPLISLPKKGSLVVYFPQGHLEQLSDYPAVAYDLPPHVFCRVVDVKLHAEVVTDEVYAQVSLVPETKQIKQKLQEGEIEADGGEEEDIEGSIKSMTPHMFCKTLTASDTSTHGGFSVPRRAAEDCFPPLDYKQQRPSQELVAKDLHGFEWRFRHIYRGQPRRHLLTTGWSAFVNKKKLVSGDAVLFLRGGDGELRLGIRRAAQIKGSSPFPALCSQQLNLNTLTAVVNAISTRSVFNICYNPRASSSEFIIPLRKFSKSIDHSFSAGMRFKMRVETEDAAERRYTGLITGISDMDPVRWPGSKWRCLLVRWDDIEANRHNRVSPWEIELSGSLSGSGSLTVPGSKRTRIGLPGTRPDFSVPNGMGVSDFGESSRFQKVLQGQEIFGFNTPYDGVDTQDHHPSEIRCFPGSSCSGIAAIGNGVRNPLGNSDISYKGIGFGESFRFHKVLQGQETFPSPPCGRALSANQAHENGSFGIFDGVQVPTSRNGWPALVQGYNAHTHLSTPSVQVSSPSSVLMFQQASTAAPNIYSMHSANNQEKEQEISNRSSFDIPEVYGEKLTPSRCELSVRGGGQGGMNFFGLLNEHNQLAVPHPLVTQSAFRGSQDLVPTCKSSCRLFGFSLTEERSIGNKVDNPTPVTSSLIPGTSFLPQQLHSEPPVMTKAIGSNCTKRTAVVRSKLQFHKLGSVVDQAINRWKLDRHDDLICALKHLFDMEGGLLHGEGKLFTRIMRML

SEQ ID NO: 12 - DNA, 2127 bp, Malus domestica
atggcgggtctaattgatctgaacagtgcgacggaggacgaggaaacgccatcgtccggctcgccgtcttcggcttcctctgtttccgacgctctgggttcgtcggcgtcggtgtgcatggagctctggcacgcctgcgcgggcccactgatttcgctgccgaagaaagggagtgtggtggtgtatctgccgcagggccacctggagcaagtctcggattttccgacctcggcttatgatctcccgccccacctcttctgtcgggttgtcgatgtcaagctccatgctgagactggcactgacgatgtcttcgctcrggtttcccttgttcctgaaagtgaggaaattgagcacagattgcgggaaggggtaaccgatgcagatgccgaggaggacgttgaggcaatggggacgtcaaccacaccccacatgttctgcaaaacccttactgcttctgatactagcactcacggaggcttctctgtgcctcgtcgtgctgccgaggattgctttcctcccctggattacactcaacaaaggccttcacaagagcttgtagcaaaggatctgcatggcctggagtggaggttccggcatatctatagggggcagccgcggaggcatttgctcaccactgggtggagtgcgtttgtgaacaagaagaagctcgtctctggagatgcagtgctgtttcttaggggtgacgatggagaactgaggctaggaattagaagggcagcccagtttaaaagttctgctacttgtccaactctttgtagccagcaattgaactatagcactatcactgatgtggtgaatgctatattcgcgaagaatgcttttaatgtgtactacaatccaaggtccagctcttctgaattcataataccttcccataagtttttgaggagccttgatcattgtttttgtgctggaatgaggatcaaaatgcgttttgaaactgaagatgcagcagagcgaagatacactgggttgataacggggattagtgaattggatcctgtaagatggcctggttcaaaatggagatgcctagttgtcaggtgggatgatrtagacacaagcaagcatggcagggtttccccatgggaagttgagcgatctggttctgtttctagttcccataccctaatgacaactggcttgaagcggtccaggattggcttgtctgcaacaaaaccagaatktccagytcctagtatgtcctgcaatyatgggattggaacatcagactttggggaatctttaaggttccagaaggtcttgcaaggtcaagaaatttcggggtttgatactcctttcagtggtttaggtggtctgaattcgcatccatctgaagcaaggagagtcttccacggttccggtggttctgggattgctgctggrggtaatggtctcagacagtcacttgtggattctgagattgcctcaaaaggcataggctttggtgaatcattccgattccataaggtcttgcaaggtcaagaaatatttccaagctcaccatatggaagagctcccgcttctaatgaagctcatgaatatggtggacctggactctatgatggttttcaggtgcctggctttaggaatggatgstccaccatgatgcagagcaataatacaaatgtgcactcatctgccccatctgtgcaagtttcatcaccttcgtctgtgttaatgttccagcaagcaatgaatccagttgcggaattcaactcggtatacaatggccataaccaagaggaccatagagtaaatcggactccacatgtcttggaacatgatggtggaaggcaaacatcatcctcattcggtgaacgtaacttcagcagggaagatcgtggaggcacacattcttacaatcagcatggtatttcacctcatccagttataagtcaatcaacaattagtggcagccaggattctgtttcaccaatcaaaggtagctgtagactctttggtttctcattgtccgaggacaaatgtgtcccggatcaagagggcaaccccaatgttggagtgcagtttcattcaaagcctcctttgatgacctcaacagttggaataacctgtactaaagtaagcaacctctttgctgcatga

SEQ ID NO: 13 - DNA, 5500 bp, Malus domestica
actctcccacgatacccacctagcaaatgctaaattytctcgctccccaaatgttctgcaatcaggcaggcargggtttagtaattagtcgggtcaaagactcggatacactaatttcaaaataaagaaatgttatagatcggagkattgtgccttggcagacaagccctctttcaacaggkttacatatgagggwtaagcaatattaaatatagattctacaaacttttgttctcaaagctgaattaacaatacaaatcaaagtcccctggagcgcttagttacaacttctgcctcaaaattaagttacataaatgacagcacacacataatcccgaagaaaacctccgcctgtcgagagttttcttcatcggtacaacgcaaaactattgatattacagtaacatcgcctgccaaaagcgaaattcaaacaaataaatgaccggaacacaagcatcttcttcatgttcatccggtttacttaaaacgactttggaaggatatagtgcggcgacaaacatggccatgatgagttccatgggtagggtttataagcggacttcraggcataccatatgtaagttttgacaatagacgggcaatgaagaatgccatgtagattccgatgctaggttgcaaacagaacaaaaatagrcaaatacaataagtaaacgtacgaggacttactagttactgcctcggatcatctgcaacaagcacaggatgatcactatccttgtaaacagctttccatcctttctccgcgccagtcaaaagcccaatcctagacataaacatcccacttgctaatcagataatcatttgcttccgtcaaatagaagattaaataccccagtcgtaacatttgaaaattgtatttcatgcagcaaagaggttgcttactttagtacaggttattccaactgttgaggtcatcaaaggaggctttgaatgaaactgcactccaacattggggttgccctcttgatccgggacacatttgtcctcggacaatgagaaaccaaagagtctacagctacctttgattggtgaaacagaatcctggctgccactaattgttgattgacttataactggatgaggtgaaataccatgctgattgtaagaatgtgtgcctccacgatcttccctgctgaagttacgttcaccgaatgaggatgatgtttgccttccaccatcatgttccaagacatgtggagtccgatttactctatggtcctcttggttatggccattgtataccgagttgaattccgcaactggattcattgcttgctggaacattaacacagacgaaggtgatgaaacttgcacagatggggcagatgagtgcacatttgtattattgctctgcatcatggtggascatccattcctaaagccaggcacctgaaaaccatcatagagtccaggtccaccatattcatgagcttcattagaagcgggagctcttccatatggtgagcttggaaatatttcttgaccttgcaagaccttatggaatcggaatgattcaccaaagcctatgccttttgaggcaatctcagaatccacaagtgactgtctgagaccattaccyccagcagcaatcccagaaccaccggaaccgtggaagactctccttgcttcagatggatgcgaattcagaccacctaaaccactgaaaggagtatcaaaccccgaaatttcttgaccttgcaagaccttctggaaccttaaagattccccaaagtctgatgttccaatcccatctgaaaaggaaacactcaaataaatcaattatgttgcagagaccagtgttatgatgacatgtcgtggtacrattgcaggacatactaggarctggamattctggttttgttgcagacaagccaatcctggaccgcttcaagccagttgtcattagggtatgggaactagaaacagaaccagatcgctcaacttcccatggggaaaccctgccatgcttgcttgtgtctayatcatcccacctgacctgcaatagcaaaagaaatgttcaaacctatatatctagtgctaatggcatgagcgaataccggaagtcaatatggacatgctacagaatagaggaaacatagtttatgatatttaggtaaacgactttcaagacagtgaaaattaactctcactatcaagacataattgctcataaaccctgagtttctactccgtaggactatgagtagggtggcttgatcaacaattaagataaaactgtgtagctaatgcgggagaaaatttatgcttccagtttaaatttagccagaaattctaccaaattgtgacatttcacatgacatatgaagtgtgcaattcatcctagttagaatacggtgaagccggctacattttttttgttaccttttgcactctcatgcttcaactattgttgagaaaagcttatcatagatttgttcatgacaatggttttgggaatctcaaagtaaaataaccaatacgtatagtaagtctcccataaagaagataatacagaatttatggtacgctaaagataacttttggtttagtacattggcattcaccacccgaaccttctcaagcagatacttataagtgcaaacaaaggggaaaaaatagtacataaaagttttgtgtagaaaatacgtacaactaggcatctccattttgaaccaggccatcttacaggatccaattcactaatccccgttatcaacccagtgtatctgccaaaaagaaaaatttaataaaaattttgcacaaaactacttcaactatttcaaaagtaagaatgccaaaccttcgctctgctgcatcttcagtttcaaaacgcattttgatcctcattccagcacaaaaacaatgatcaaggctcctcaaaaacttatgggaaggtattatgaattcagaagagctggacctacaagatcatggacgattataaggaaaaaagatgcagaaggaagaaaggtctaaagtctcaagcacgataactttcaacattactttaggaacatgttaaatgatgagcaccagattaccttggattgtagtacacattaaaagcattcttcgcgaatatagcattcaccacatcagtgatagtgctatagttcaattgctggctacaaagagttggacaagtagcagaacttttaaactgggctgcccttctaattcctagcctcagttctccatcgtcacccctattataaatactggatgagaattataaatawggggatccaaaatctcttcaatcgaagggtttatatacctaagaaacagcactgcatctccagagacgagcttcttcttgttcacaaacgcactccacccagtggtgagcaaatgcctccgcggctgccctactcaaaccaattagaaaaaaggaataagaaacagaaaaacgttgaatctaaagcatccaatttacaaagttcattataaaactctaataagattgctaccgtatcatggaaagataaacccccaactaatgaagcacaaaagggatcatattttttgtattacccctatagatatgccggaacctccactccaggccatgcagatcctttgctacaagctcttgtgaaggcctttgttgagtgtaatcctaaaagcacaatctattcgtctcaaaaacaaaatactaatatgtacttgattagactaataatttagtctcaaaaaagttatgcagaagctaaamcaaaagttgggggagaacatgaactaggaataccaggggaggaaagcaatcctcggcagcacgacgaggcacagagaagcctccgtgagtgctagtatcagaagcagtaagggttttgcagaacatgtggggtgtggttgacgtccccattgcctcaacgtcctcctcggcatctgcatcggttaccccttcccgcaatctgtgctcaatttcctacaccgattaaagcattagtgaaatcacctcaatgtcaatgtttaacagacaaaaacatcacamgatcaccaggaagagcaaagaaaattaaaaaacaycaaccccgaaatcgaattgtataaattataagtaactaattcataaatttgtgaaatgactaattgtaaggaracagagatgctaacatataatcttcgataatgccaaagtgggaaagaaagaaagtgaaattctaaagcttgcgtttttaattgtttcggtttctacggaaagggaggattttctcagaatttttttacttttcgagcattttctcaggaaccaaacaaaaaatcaaaccttgtacaaataaacccacctcactttcaggaacaagggaaaccygagcgaagacatcgtcagtgccagtctcagcctgcgaccaaaaaagacctcaagaaattgagaacccagatagcaaaaccccaaaagctatcaaatttcatcaaaaatccaaaaccccaaaagcatggagaaagagaggctcattgtatagagagagactgacatggagcttgacatcgacaacccgacagaagaggtggggcgggagatcataagccgaggtcggaaaatccgagacttgctccaggtggccctgcggcagatacaccaccacactccctttcttcggcagcgaaatcagtgggcccgcgcaggcgtgccagagctccatgcacaccgacgccgacgaacccagagcgtcggaaacagaggaagccgaagacggcgagccggacgatggcgtttcctcgtcctccgtcgcactgttcagatcaattagacccgccatgtgaaattaaacagaaactgtaaggacccaacaagcgaaagaggaagaagaaggagaaaagcactttgcttttttgctttttgcttctgcttctgcttaagcttgtttataatatggagaagagaaaaaaragagcagatgaggtttcaattctcctgcattttgagagatgggtttgatggcatttttgctaaaagaagctcagaaaagcacttctctctcttttctgcttaattcttaacttttatttatttttcttttggacgggcttttgggtatcaaatcaaaagctcaaagcttttacaatttgggagatgagaaaaagaaaatggaaattaataccaaaaaaaatcagataatttaatatgggacttcttttggtgttgaattgaatccctttttgggtttttaaattacaaaagattaaaccttttctctctgtctgcaggctgaactgcaacactgcaattgctgggtgtgatgtgtggcagaaacagtgtgtcagagagtgagagagagaggaagagagagagtggaggtcttgtacggcaccccctgtatttccgggcggatgtctattctgtccccttctactccgtcaaatcccactcgtatccccccccccctcttccttaatcttcattctctccttcctcccatatttaatttattttaattaaggaggatgtagttaaactaagattttaaaagatttt

SEQ ID NO: 14 - DNA, 2127 bp, Malus domestica
atggcgggtctaattgatctgaacagtgcgacggaggacgaggaaacgccatcgtccggctcgccgtcttcggcttcctctgtttccgacgctctgggttcgtcggcgtcggtgtgcatggagctctggcacgcctgcgcgggcccactgatttcgctgccgaagaaagggagtgtggtggtgtatctgccgcagggccacctggagcaagtcttggattttccgacctcggcttatgatctcccgccccacctcttctgtcgggttgtcgatgtcaagctccatgctgagactggcactgacgatgtcttcgctcrggtttcccttgttcctgaaagtgaggaaattgagcacagattgcgggaaggggtaaccgatgcagatgccgaggaggacgttgaggcaatggggacgtcaaccacaccccacatgttctgcaaaacccttactgcttctgatactagcactcacggaggcttctctgtgcctcgtcgtgctgccgaggattgctttcctcccctggattacactcaacaaaggccttcacaagagcttgtagcaaaggatctgcatggcctggagtggaggttccggcatatctatagggggcagccgcggaggcatttgctcaccactgggtggagtgcgtttgtgaacaagaagaagctcgtctctggagatgcagtgctgtttcttaggggtgacgatggagaactgaggctaggaattagaagggcagcccagtttaaaagttctgctacttgtccaactctttgtagccagcaattgaactatagcactatcactgatgtggtgaatgctatattcgcgaagaatgcttttaatgtgtactacaatccaaggtccagctcttctgaattcataataccttcccataagtttttgaggagccttgatcattgtttttgtgctggaatgaggatcaaaatgcgttttgaaactgaagatgcagcagagcgaagatacactgggttgataacggggattagtgaattggatcctgtaagatggcctggttcaaaatggagatgcctagttgtcaggtgggatgatrtagacacaagcaagcatggcagggtttccccatgggaagttgagcgatctggttctgtttctagttcccataccctaatgacaactggcttgaagcggtccaggattggcttgtctgcaacaaaaccagaatktccagytcctagtatgtcctgcaatyatgggattggaacatcagactttggggaatctttaaggttccagaaggtcttgcaaggtcaagaaatttcggggtttgatactcctttcagtggtttaggtggtctgaattcgcatccatctgaagcaaggagagtcttccacggttccggtggttctgggattgctgctggrggtaatggtctcagacagtcacttgtggattctgagattgcctcaaaaggcataggctttggtgaatcattccgattccataaggtcttgcaaggtcaagaaatatttccaagctcaccatatggaagagctcccgcttctaatgaagctcatgaatatggtggacctggactctatgatggttttcaggtgcctggctttaggaatggatgstccaccatgatgcagagcaataatacaaatgtgcactcatctgccccatctgtgcaagtttcatcaccttcgtctgtgttaatgttccagcaagcaatgaatccagttgcggaattcaactcggtatacaatggccataaccaagaggaccatagagtaaatcggactccacatgtcttggaacatgatggtggaaggcaaacatcatcctcattcggtgaacgtaacttcagcagggaagatcgtggaggcacacattcttacaatcagcatggtatttcacctcatccagttataagtcaatcaacaattagtggcagccaggattctgtttcaccaatcaaaggtagctgtagactctttggtttctcattgtccgaggacaaatgtgtcccggatcaagagggcaaccccaatgttggagtgcagtttcattcaaagcctcctttgatgacctcaacagttggaataacctgtactaaagtaagcaacctctttgctgcatga

SEQ ID NO: 15 - DNA, 5500 bp, Malus domestica
aaaatcttttaaaatcttagtttaactacatcctccttaattaaaataaattaaatatgggaggaaggagagaatgaagattaaggaagagggggggggggatacgagtgggatttgacggagtagaaggggacagaatagacatccgcccggaaatacagggggtgccgtacaagacctccactctctctcttcctctctctctcactctctgacacactgtttctgccacacatcacacccagcaattgcagtgttgcagttcagcctgcagacagagagaaaaggtttaatcttttgtaatttaaaaacccaaaaagggattcaattcaacaccaaaagaagtcccatattaaattatctgattttttttggtattaatttccattttctttttctcatctcccaaattgtaaaagctttgagcttttgatttgatacccaaaagcccgtccaaaagaaaaataaataaaagttaagaattaagcagaaaagagagagaagtgcttttctgagcttcttttagcaaaaatgccatcaaacccatctctcaaaatgcaggagaattgaaacctcatctgctctyttttttctcttctccatattataaacaagcttaagcagaagcagaagcaaaaagcaaaaaagcaaagtgcttttctccttcttcttcctctttcgcttgttgggtccttacagtttctgtttaatttcacatggcgggtctaattgatctgaacagtgcgacggaggacgaggaaacgccatcgtccggctcgccgtcttcggcttcctctgtttccgacgctctgggttcgtcggcgtcggtgtgcatggagctctggcacgcctgcgcgggcccactgatttcgctgccgaagaaagggagtgtggtggtgtatctgccgcagggccacctggagcaagtcttggattttccgacctcggcttatgatctcccgccccacctcttctgtcgggttgtcgatgtcaagctccatgtcagtctctctctatacaatgagcctctctttctccatgcttttggggttttggatttttgatgaaatttgatagcttttggggttttgctatctgggttctcaatttcttgaggtcttttttggtcgcaggctgagactggcactgacgatgtcttcgctcrggtttcccttgttcctgaaagtgaggtgggtttatttgtacaaggtttgattttttgtttggttcctgagaaaatgctcgaaaagtaaaaaaattctgagaaaatcctccctttccgtagaaaccgaaacaattaaaaacgcaagctttagaatttcactttctttctttcccactttggcattatcgaagattatatgttagcatctctgtytccttacaattagtcatttcacaaatttatgaattagttacttataatttatacaattcgatttcggggttgrtgttttttaattttctttgctcttcctggtgatcktgtgatgtttttgtctgttaaacattgacattgaggtgatttcactaatgctttaatcggtgtaggaaattgagcacagattgcgggaaggggtaaccgatgcagatgccgaggaggacgttgaggcaatggggacgtcaaccacaccccacatgttctgcaaaacccttactgcttctgatactagcactcacggaggcttctctgtgcctcgtcgtgctgccgaggattgctttcctcccctggtattcctagttcatgttctcccccaacttttgktttagcttctgcataacttttttgagactaaattattagtctaatcaagtacatattagtattttgtttttgagacgaatagattgtgcttttaggattacactcaacaaaggccttcacaagagcttgtagcaaaggatctgcatggcctggagtggaggttccggcatatctataggggtaatacaaaaaatatgatcccttttgtgcttcattagttgggggtttatctttccatgatacggtagcaatcttattagagttttataatgaactttgtaaattggatgctttagattcaacgtttttctgtttcttattccttttttctaattggtttgagtagggcagccgcggaggcatttgctcaccactgggtggagtgcgtttgtgaacaagaagaagctcgtctctggagatgcagtgctgtttcttaggtatataaacccttcgattgaagagattttggatccccwtatttataattctcatccagtatttataataggggtgacgatggagaactgaggctaggaattagaagggcagcccagtttaaaagttctgctacttgtccaactctttgtagccagcaattgaactatagcactatcactgatgtggtgaatgctatattcgcgaagaatgcttttaatgtgtactacaatccaaggtaatctggtgctcatcatttaacatgttcctaaagtaatgttgaaagttatcgtgcttgagactttagacctttcttccttctgcatcttttttccttataatcgtccatgatcttgtaggtccagctcttctgaattcataataccttcccataagtttttgaggagccttgatcattgtttttgtgctggaatgaggatcaaaatgcgttttgaaactgaagatgcagcagagcgaaggtttggcattcttacttttgaaatagttgaagtagttttgtgcaaaatttttattaaatttttctttttggcagatacactgggttgataacggggattagtgaattggatcctgtaagatggcctggttcaaaatggagatgcctagttgtacgtattttctacacaaaacttttatgtactattttttcccctttgtttgcacttataagtatctgcttgagaaggttcgggtggtgaatgccaatgtactaaaccaaaagttatctttagcgtaccataaattctgtattatcttctttatgggagacttactatacgtattggttattttactttgagattcccaaaaccattgtcatgaacaaatctatgataagcttttctcaacaatagttgaagcatgagagtgcaaaaggtaacaaaaaaaatgtagccggcttcaccgtattctaactaggatgaattgcacacttcatatgtcatgtgaaatgtcacaatttggtagaatttctggctaaatttaaactggaagcataaattttctcccgcattagctacacagttttatcttaattgttgatcaagccaccctactcatagtcctacggagtagaaactcagggtttatgagcaattatgtcttgatagtgagagttaattttcactgtcttgaaagtcgtttacctaaatatcataaactatgtttcctctattctgtagcatgtccatattgacttccggtattcgctcatgccattagcactagatatataggtttgaacatttcttttgctattgcaggtcaggtgggatgatrtagacacaagcaagcatggcagggtttccccatgggaagttgagcgatctggttctgtttctagttcccataccctaatgacaactggcttgaagcggtccaggattggcttgtctgcaacaaaaccagaatktccagytcctagtatgtcctgcaatygtaccacgacatgtcatcataacactggtctctgcaacataattgatttatttgagtgtttccttttcagatgggattggaacatcagactttggggaatctttaaggttccagaaggtcttgcaaggtcaagaaatttcggggtttgatactcctttcagtggtttaggtggtctgaattcgcatccatctgaagcaaggagagtcttccacggttccggtggttctgggattgctgctggrggtaatggtctcagacagtcacttgtggattctgagattgcctcaaaaggcataggctttggtgaatcattccgattccataaggtcttgcaaggtcaagaaatatttccaagctcaccatatggaagagctcccgcttctaatgaagctcatgaatatggtggacctggactctatgatggttttcaggtgcctggctttaggaatggatgstccaccatgatgcagagcaataatacaaatgtgcactcatctgccccatctgtgcaagtttcatcaccttcgtctgtgttaatgttccagcaagcaatgaatccagttgcggaattcaactcggtatacaatggccataaccaagaggaccatagagtaaatcggactccacatgtcttggaacatgatggtggaaggcaaacatcatcctcattcggtgaacgtaacttcagcagggaagatcgtggaggcacacattcttacaatcagcatggtatttcacctcatccagttataagtcaatcaacaattagtggcagccaggattctgtttcaccaatcaaaggtagctgtagactctttggtttctcattgtccgaggacaaatgtgtcccggatcaagagggcaaccccaatgttggagtgcagtttcattcaaagcctcctttgatgacctcaacagttggaataacctgtactaaagtaagcaacctctttgctgcatgaaatacaattttcaaatgttacgactggggtatttaatcttctatttgacggaagcaaatgattatctgattagcaagtgggatgtttatgtctaggattgggcttttgactggcgcggagaaaggatggaaagctgtttacaaggatagtgatcatcctgtgcttgttgcagatgatccgaggcagtaactagtaagtcctcgtacgtttacttattgtatttgyctatttttgttctgtttgcaacctagcatcggaatctacatggcattcttcattgcccgtctattgtcaaaacttacatatggtatgcctygaagtccgcttataaaccctacccatggaactcatcatggccatgtttgtcgccgcactatatccttccaaagtcgttttaagtaaaccggatgaacatgaagaagatgcttgtgttccggtcatttatttgtttgaatttcgcttttggcaggcgatgttactgtaatatcaatagttttgcgttgtaccgatgaagaaaactctcgacaggcggaggttttcttcgggattatgtgtgtgctgtcatttatgtaacttaattttgaggcagaagttgtaactaagcgctccaggggactttgatttgtattgttaattcagctttgagaacaaaagtttgtagaatctatatttaatattgcttawccctcatatgtaamcctgttgaaagagggcttgtctgccaaggcacaatmctccgatctataacatttctttattttgaaattagtgtatccgagtctttgacccgactaattactaaacccytgcctgcctgattgcagaacatttggggagcgagaraatttagcatttgctaggtgggtatcgtgggagagt

SEQ ID NO: 16 - DNA, 2367 bp, Arabidopsis thaliana
taatgtctctctctccacgcacaaaaggtctaaaagccacaccacacacatcagtcaccagacgtagcagagagcctcactgttgcagagagcactcagtactgttctgtttctctgatacctctctctctcctctctcttttaacattgtccaaattaaaaatctaaactttttttctagttttttttttttctttaatagaaaagttttttttctccacggcttaaagactcactcatcactgtgctactactctctcttcttttggctgagagggtaaaagtcatgaagaaactcctctgagttttttttctttctttcttataataaagctcttatctttatctctgtttctctctctttaatgggtggtttaatcgatctgaacgtgatggagacggaggaagacgaaacgcaaacgcaaacaccgtcttcagcttctgggtctgtctctcctacttcgtcttcttcagcttctgtgtctgtggtgtcttcgaattctgctggtggaggggtttgtttggagctgtggcatgcttgtgctggaccccttatctctctaccaaaaagaggaagccttgtgttgtatttccctcagggacatttggaacaagcccccgatttctccgccgcgatttacgggctccctcctcacgtgttctgtcgtattctcgatgttaagcttcacgcagagacgactacagatgaagtttatgctcaagtctctcttcttcctgagtcagaggacattgagaggaaggtgcgtgaaggaattatagatgttgatggtggagaggaagattatgaagtgcttaagaggtctaatactcctcacatgttttgcaaaacccttactgcttctgatacaagcacccatggtggtttctctgttcctcgccgagctgctgaggattgcttccctcctctggactatagccagccccggccttctcaggagcttcttgctagggatcttcatggcctggagtggcgatttcgccacatttatcgagggcaacctaggaggcatttgctcactaccgggtggagtgcgtttgtgaacaagaagaagcttgtctctggtgatgctgtgcttttccttagaggagatgatggcaaactgcgactgggagttagaagagcttctcaaatcgaaggcaccgctgctctctcggctcaatataatcagaatatgaaccacaacaatttctctgaagtagctcatgccatatcgacccatagcgttttcagcatttcctacaaccccaaggcaagctggtcaaacttcataatccctgcaccaaagttcttgaaggttgttgactatcccttttgcattgggatgagatttaaagcgagggttgaatctgaagatgcatctgagagaagatcccctgggattataagtggtatcagcgacttggatccaatcaggtggcctggttcaaaatggagatgccttttggtaaggtgggacgacattgtggcaaatgggcatcaacagcgtgtctcgccatgggagatcgaaccatctggttccatctccaattcaggcagcttcgtaacaactggtcccaagagaagcaggattggcttttcctcaggaaagcctgatatccctgtctctgaggggattcgcgccacagactttgaggaatcattgagattccagagggtcttgcaaggtcaagaaatttttccgggttttatcaacacttgttcggatggtggagccggtgccaggagaggccgcttcaaaggaacagaatttggtgactcttatggtttccataaggtcttgcaaggtcaagaaacagttcccgcctactcaataaccgatcatcggcagcagcacgggttgagccagaggaacatttggtgtgggccgttccagaactttagtacacgtatcctccccccatctgtatcatcatcaccctcttccgtcttgcttaccaactcgaacagtcctaacggacgtctggaagaccatcacggaggttcaggcagatgcaggctgtttggtttcccattaaccgacgaaaccacagcagttgcatctgcgacggctgtcccctgcgttgaagggaattccatgaaaggtgcgtcagctgttcaaagcaatcatcatcattcgcaaggaagggacatctatgcaatgagagacatgttgctagacattgctctctagaagggttctttggtttctgtgttttatttgcttgtggcttaagtaaagttcttattttagttgatgatgacttgctgctaacttttggaatgtcacaagttgtgacttatgagagacttgtaaacttggttcaagaatgttctgtgttaggttcaatttaaaaagtgtttgcatc

SEQ ID NO: 17 - DNA, 3710 bp, Arabidopsis thaliana
taatgtctctctctccacgcacaaaaggtctaaaagccacaccacacacatcagtcaccagacgtagcagagagcctcactgttgcagagagcactcagtactgttctgtttctctgatacctctctctctcctctctcttttaacattgtccaaattaaaaatctaaactttttttctagttttttttttttctttaatagaaaagttttttttctccacggcttaaagactcactcatcactgtgctactactctctcttcttttggctgagagggtaaaagtcatgaagaaactcctctgagttttttttctttctttcttataataaagctcttatctttatctctgtttctctctctttaatgggtggtttaatcgatctgaacgtgatggagacggaggaagacgaaacgcaaacgcaaacaccgtcttcagcttctgggtctgtctctcctacttcgtcttcttcagcttctgtgtctgtggtgtcttcgaattctgctggtggaggggtttgtttggagctgtggcatgcttgtgctggaccccttatctctctaccaaaaagaggaagccttgtgttgtatttccctcagggacatttggaacaagcccccgatttctccgccgcgatttacgggctccctcctcacgtgttctgtcgtattctcgatgttaagcttcacgtatgtaactaactctctctttctttctattttttgttttgttttgttttcttcatttatgttttctcctctgctctcaaagcagagagatatgggttttgttctgtttttctgattctttgatttttttaattgtttgtttggtgaatctgagttgggttttcgatacaagtatggagatttgtgcctttggtttattgaattgtttgagacaaacgaatttatgttgggagaaaagtttcctcttttgctccatttgcatttcttctcgtggcattttgatgacgaatacttgaaatccccataaattatcttcagttttttctttgatgataatgaatttgatttcaaagtttcgccttttgctccattttgatgacaattgatttcagaacaattcaattctctgtaaaggtttaaactttttttgttgttgtgaggattaataaacaaaatgtgggggattttgatttcgtaggcagagacgactacagatgaagtttatgctcaagtctctcttcttcctgagtcagaggtgagtttttctttaggctcttgagttttgtaacaaagagagagaaatttgctcgagcttagggggtttgagttgatttgttacaggacattgagaggaaggtgcgtgaaggaattatagatgttgatggtggagaggaagattatgaagtgcttaagaggtctaatactcctcacatgttttgcaaaacccttactgcttctgatacaagcacccatggtggtttctctgttcctcgccgagctgctgaggattgcttccctcctctggtactaatccactctctgtagattctgtaatcagctttgtacattgcacattgtgttctagagttctcttattagctcatattgagagattttaactacataatcattttgttatgtaggactatagccagccccggccttctcaggagcttcttgctagggatcttcatggcctggagtggcgatttcgccacatttatcgaggtaagtttgttgccttatgttgcaatttttcttgcctggatttagtagatggaaaatttgaatggtttgagtgacttttagggcaacctaggaggcatttgctcactaccgggtggagtgcgtttgtgaacaagaagaagcttgtctctggtgatgctgtgcttttccttaggtagttaaaaatgcttctatgttttctcactacacaacctctttgattttctgtaagaggttttgtgatatatgggtttctctgatacagaggagatgatggcaaactgcgactgggagttagaagagcttctcaaatcgaaggcaccgctgctctctcggctcaatataatcagaatatgaaccacaacaatttctctgaagtagctcatgccatatcgacccatagcgttttcagcatttcctacaaccccaagtaagccccaaccacaatgaccttttttcgttttcagcatttaaaatttcatttcagaatcataattagaatctcctgaagccttaagttgtgtattgttctagttgattgttccttagaagtttgttaactccaataaatatcaggaatttagcattaatactagttcactggtaaaacattttcagggcaagctggtcaaacttcataatccctgcaccaaagttcttgaaggttgttgactatcccttttgcattgggatgagatttaaagcgagggttgaatctgaagatgcatctgagagaaggttacttatagacttataattcaagctttaagataaccttgcacacctgtgttttatatgcccaactttctaacatgtttcacctgttttgtcagatcccctgggattataagtggtatcagcgacttggatccaatcaggtggcctggttcaaaatggagatgccttttggtaagctatgaattatgttcttaagtcattagtttggtctgagaggtcttctataagattgttgccttttctatatccgtaagctcactgctctgaaactatgttttgacgtcatattcaggtaaggtgggacgacattgtggcaaatgggcatcaacagcgtgtctcgccatgggagatcgaaccatctggttccatctccaattcaggcagcttcgtaacaactggtcccaagagaagcaggattggcttttcctcaggaaagcctgatatccctgtctctggtacacatctacttagccaaagacattgtaccactcatataaccatttatcgcctgtaatataacgttttctgctattattgcagaggggattcgcgccacagactttgaggaatcattgagattccagagggtcttgcaaggtcaagaaatttttccgggttttatcaacacttgttcggatggtggagccggtgccaggagaggccgcttcaaaggaacagaatttggtgactcttatggtttccataaggtcttgcaaggtcaagaaacagttcccgcctactcaataaccgatcatcggcagcagcacgggttgagccagaggaacatttggtgtgggccgttccagaactttagtacacgtatcctccccccatctgtatcatcatcaccctcttccgtcttgcttaccaactcgaacagtcctaacggacgtctggaagaccatcacggaggttcaggcagatgcaggctgtttggtttcccattaaccgacgaaaccacagcagttgcatctgcgacggctgtcccctgcgttgaagggaattccatgaaaggtgcgtcagctgttcaaagcaatcatcatcattcgcaaggaagggacatctatgcaatgagagacatgttgctagacattgctctctagaagggttctttggtttctgtgttttatttgcttgtggcttaagtaaagttcttattttagttgatgatgacttgctgctaacttttggaatgtcacaagttgtgacttatgagagacttgtaaacttggttcaagaatgttctgtgttaggttcaatttaaaaagtgtttgcatc

SEQ ID NO: 18 - DNA, 2935 bp, Phaseolus vulgaris
ccatgataaaataacattttgcttgtgaaatgttactggttgttttggttacatccaacttcattgatggtgtcagtgttctgtaagtgagaaaattgaattttggagtggtttggttaagagagatggttaaatgtggaggataacggtagagtgagttggtaagagagtgggaatgaaagggtttcccaaaaagcgaaccccataattgtgtgaggagtgaagagcccaaaaagggtgggaaaaatgaagagagagtgattggtcagtgggagagaaagacagagacagagaaagcgggtctctttctttttggagtattgggtcaggttcttttggcaatgccaaagttggtcacgctctctgaaaatgcaggaggcatgaaaccactccttcaaatatctcccaccactcactcgctcctgtgctgcttcttcttctccttctgtttctgttccttctctctctatctccctcttttctcctcctcctcctcatgcctgccctcatcgatctcaacagcgccaccgaggaccatgaaacgccgtcgtctcgcccatcctccgtctgcctcgaactctggcacgcctgcgcgggtcctatgatctccttgcccaagaaagggacccttgtcgtgtacttccctcaaggacacttggaacaacaccttcacgattttccgctccctgcttctgctaacatcccctcccatctcttctgtcgcgttctcgatgtcaagctccattctgaggaagggagcgatgaggtgtattgccaggtggtgctggttcccgaaagtgagcaagggcatcagaagttgcgggaaggggaaattgatgctgatggtgaagaggaggatgctgaagctgtgatgaagtccaccacaccccacatgttctgcaagactttgacagcttctgatactagcactcatggcggattctctgtgcctcgtcgtgctgcggaagattgttttccacctctggattacagtcaacagagaccttcacaggagcttgtggcgaaggatctgcatggccaagaatggaggttccgacatatttatagggggcaaccacgacgacacttgcttaccactgggtggagtgcatttgtgaacaagaagaaacttgtatctagagatgctgttctgtttcttaggggtgaggatggagaactgagattgggaattcgtagggctgctcaattgaaaagtggcagtaccatttcaacttttgctggccagcaattgaatcatagcagtcttctggatgtggttaatgctttatcagcaagatgtgcctttagtgttcactataatccaagggtcagttcatctgagttcatcatacccattaagaaattcttgaggagccttgattattcttattcagttggaacaagatttaggatgcgttttgaaactgaagatgctgcagagcgaagatttacaggattgattgttggaattactgatgtggatcctgttagatggcctggatcaaaatggagatgcctaatggtaaggtgggatgacctggaagccacaaggcataatagggtttcaccctgggagattgagccatctggttctgcatctactgcaaataacatgatatcagctggtttgaagaggaccaagattggattgccttcaaccaagctagattttcaagtttccaatgcaattggagcatcagactttggcgaatcactaaggttccagaaggtcttgcaaggtcaagaaatgttgggtgttaacacaacttttgatagtactaatggtcagggtcaccagctatcagatttgaggagatgctatcctggctcaaactgttctaggattgctgcaaccggaaacagcattggaattccgcaagtgagttccaatgtttcctgcaatggcataggcttcagtgaatctttcagattccagaaggtcttgcaaggtcaagaaatacttccaagccaaccatatggaagggccctgtctgttgatgaggcttgtggaaatggtcgctttggaccttttgatggttaccatacactgagatccagaaatggatggtcttcccacttgagtaacagttcttcacatttgcatccacctgttccatctgggcaagtttcatctccatcatctgtgttaatgttccagcaagcacacaatccagtttcaaactctgattacaacagcaaaattagtcaggtgatggaaggtaaagtccagcaacgatcatcatacacttctgaagctaaaggtggaaaatttgtatcaaccccttatgagcctcttcgtggactagctcaggaaggcacaaattcttatggggtctcaaacttgcacaatcagtttgaaacttcacgttcacacgattctatttcagcacttcgggctactcaagagttggttcccacatgtaaaagtcgatgcagagtctttggcttctcattaactgagggtgctcctgttgcaagtaaagaagtagccggcaccgacccatcggccgtcacatgttctggaccttcctttgcaagacacgctgaagatgatttccatccagtgcatagcaaggcagtgggaagttattgcaccaaaggtgtgctgcaatattgacttgaaaatcatggtgtatggtagtagttatgctgtcataaggtggcagaagagaatgttcactgttgtactaatgtggagaatatgataactattcgcctaactagatatttatcttgttaaattggctgtgacacaatcaatttctgtattaatctatgtactctttattgacttgtaaaacgatgcatgtgtgttcactgttatggccatatgaggctctggtggcactgcataacccttcatttatcttgaattgggcatgattactttagggaactatagctcatcatgtttcatgaccttaagttatctcca

SEQ ID NO: 19 - DNA, 2762 bp, Lycopersicum esculentum
aattcgcccttgagtgcgcagttgaactagcaaaagggtttaaagatgatgtgtggacttattgatctgaatactgtggataacgatgatgccggagaagaaacgacggcgccggtgtcattggattcaccggcgtcgtcgtcggcggcatcaggaagttcggatttaacgtcgtcaactacgccagcggtggcatcggtgtgtatggagctttggcatgcgtgtgctggaccgttgatttcgctgccgaagaaaggaagtgcggttgtgtacctgcctcaaggtcacttggaacatttatctgagtacccgtccatagcctgtaatctccctcctcatgtgttttgtcgcgttgtagatgtgaagctacaagcagatgcggctactgatgaggtctatgcacaagtctcactagttcctgacaatcagcagattgagcagaaatggaaggatggagacattgatgctgatattgaagaagaggaaatagaaggtgctggaaaatcaataacaccacacatgttctgcaaaactcttactgcatcggataccagcactcatggtggtttctctgtccctcggcgggcagcagaagattgttttgctcccttggattacagacaacagaggccctcgcaggagctggtagccaaagatctacatggtatagagtggaaatttcggcatatctatcggggtcagccacggcggcatctgctcactacaggatggagtgcatttgtaaacaagaagaagcttgtttctggtgacgctgttcttttcttgaggactggtgatggagagcttaggttaggagtgagacgagctgcccaagcaaaaacatgttctagttatctggctccttgtagcaaaccgttgaatgttagtggcattgtagatgctgttaacgttatatctagcagaaatgctttcaacatttgttacaacccaagggatagctcatcggatttcattgtaccttaccacaaattctctaagactcttgcacatcccttttcagctggaatgaggtttaaaatgcgtgtcgaaacagaagatgcagctgagcaaaggttcactggactagttgtgggagtcagcaatgtagatccagttcgatggccaggttctaaatggaggtgcctattggtcagatgggatgatcttgatgtttctagacataatagggtttcaccatgggagattgagccatctggttcagctcctgtgcccagcagcttggtgatgccttctgctaagaggaccagggttggcttccctatttcaaaggcagattttccaattcctagagaaggaattgcagtatcagactttggggaaccttctaggttccagaaggtcttgcaaggtcaagaaattttgaggatgcatgctccttatggcggacttgatgctcggagtcctcgtccagcaggcacaagatgctttcctggttttcctagttctgggatatctagaatgggaaacagcatcagacccctgtttggtgacactgacaagtcccatgaaagcattggctttagtgaatctcttcgattcaataaggtcttgcaaggtcaagaaatttttacaagccctccttatgggagagctcaagctggtatccaaatgcaggagaaaagtaggaccggtatttttgtcggtattcaggttccaaaccatggaaacaggtggcctgctccaaatcaggataataacactccttgcaagccaattaatcctgtctcagcatcatcaccgccttctgcactcaattttcagcatccgagccctccagcatcaaagttccaggctatgttcaatcataaacatgatcttgttaaccaggcttcgttagatctgtctgagaactgttgtaggtatccgtatctctcatctggttcacataccgaggacatcagtcagaaggaaggtactcaaggaatcagctcgtttggtttcttaaaggagcaaaagcaaacaggactttcatatctttctcctgggacacagtcgtcattcaaaggcaatcaaaacttagtttccacttgtaaaactggttgcaggatctttgggttccccttgaccgagagtaaaataagtgcaactagagcggatactccctctgaagctgtatactcacatggtctagaaactacatttctcccttccagtgatggaaagttgcagccggggccaccattgatgactaacgttgtggggacaaattttaccaaagtaaatgacctctatgcagcaagagatgtgcttcttgatattgctctgtagcaggtgtttgttgtgaggttgtgctagaatatgtagactgaaggatgtgtgtgcagcattattgattattagcttttagttggcgttgtaatcttctggctgttgagtgcgcaagcatttggttgccagtagaatgcttatccagagatgagaattgagagttattaatgaagattgataccgttgaggaacgtatgttcttgaaaatttggtgtatatgttcctgtgacgctgatgtactatgtaacaattggaagctgtgtttgctgcatcaaagatgtctgtatgatagttgtactctacttgagatgacttctgtatttgtatatttacctagtctagatttgctgtgaactaactcgagctcctataaatcggtaagtttgttgtaggagctctcgtctcaggaacacaatactgtactgaattttgtaaggaattgtcatgtatattcctgcaattaagggcgaatt

SEQ ID NO: 20 - DNA, 2622 bp, Citrus clemantina
ttgacgaagttgcagcagccagcagcacttaaaacacttgcctctaaaatgcagtcatgaaactctctctccttctcgctctcaaaagcacttgtttttcacaactttttcttctcagcttccactacaacaccattgtatcgttctaagcatctctctaaaatggtgggtttgattgatcttaacacaacagaagacgatgagaatccgtcatcgggatctttatctccgtcctcttcttctgcttctgccttgagtgcttctggtttcgctttagctcctgcttctgcttctgcttctggggtgtctttagagctatggcacgcatgtgcagggccactaatatctctgcccaagagaggcagtgtggtcgtttacttccctcagggacatttggagcatgtctccgatttttccgccgctgcttcagctgcttatgatctcccccctcatctgttttgtcgggttgctgatgtcaagctccatgcagaggcggcaagtgatgaggtttatgcgcaggtctcactggttccagatgagctaattgagcagaaggtgcgtgaagggaaaattgaggaggatggtgatgaggagagtgttgaggtggttgctaagtcttcaacaccccacatgttctgcaagaccctcacggcttctgatactagcactcatggaggcttctctgtacctcgtcgagctgcagaagactgcttccctcccctggactatagtcaacagaggccttcacaggagcttgtggcaaaggatctccatggcctggaatggaggttccggcacatttacagggggcaaccacggaggcatttgctgactactggatggagtgcatttgttaataagaagaagcttgtttctggagatgctgtgcttttccttaggggtgaagatggtgaattgagacttggaatccgaagagcacctcatgtaaaaagtggtgctactttcccttctttctgcagccaacagtcgagtcccaattctgtcacagaggtggttgatgccatagctaggaagcgtgctttcagcatttcctacaatccaagggccagcgcctcagagttcataattcctgtcaataagtttttgaagagccttggtcattctttcgctgttggaatgaggttcaaaatgcgttttgaaacagaagatgcagcagagcgaagatacactggagtgattatgggagtcggtgacatggatcctgtgagatggcctggttcaaaatggagatgcctgttggtgagatgggatgatgttgagtccaacaggcacaccagggtatctccatgggaaattgagccatctggttctgtttgtggttccaataacctgatcacatctggtttgaagaggaccaggattggattgccttctgggaaaccagaatttccagttcctgatggaattggagtgacagactttggggaatctttgaggttccagaaggtcttgcaaggtcaagaaatattaggttttaacactctttatgatggtggtgattgtcagaatctgcatccatctgaagtaaggaggggcattcctggttcaaatggttctgggattgctgctataggagatggtagcagaaacctgcaggtgaaatctgacatttcctacaaaggcataggcataggctttggtgaatcattccgattccataaggtcttgcaaggtcaagaaatatttccgaagtctccatatggaagagcccctactaataatgaggctcgtagtattggcagccttggaatctctgatggtgttccggtatctggatcaagaaatagatggtctgctgtggtgccgggctataacactcatatgagcccatctgcaccgcctgtacaagtgtcatcaccttcttcggtgttaatgtttcagctggcaagcaatccaatttctaactataatcctccttatagcttgaacgatcaggagaaagagcaacgtgtcaactgtcaaagcttttttcataattctgaaatatatggaggaaagcatgcatcatcttcatttcttgaccatagtttcgtggggggtgatcaggaggtcatggattctataggtcagtcaaatgagcatatttcaccacctcttgtaggtcagccaacagttaggggcagccaagatttagtttcctcgtgtaagggtagctgcagactctttggtttttcattgactgaggaaagacatgttgccaacatagaggacaatgcagctccagttgcgtctcctttgaatcctagatcttcttttctgtctcatgttggacagcagttccatccaaagcctccagtaatgtctaaggcaactggaagcaactgtaccaatggaatcatgcaacattgtcttggaaattatgatatatactaaccaaggtgcagaggtagcacctgggcttgcagaagaaaatgcttgtaattgctctaattatacatatgctgtagtaaatgatacaatttaattagctggtgagaaaaccaagtgtaagtatttttttcaaagtaacttgatgtcatgattatgcttaactccactatggaaagcaaacaacatatgtattgtattaatctattaagtttccagcggatgttgtctatt

SEQ ID NO: 21 - DNA, 2917 bp, Fragaria vesca
ctttcactgtctttctctgccacacatcacacccagcagttgcagcgttgcagaggctgcagcactgcagcagagctgcagagagagacagactcaaagaaataatataaaaattcgcaaggaaaaagataaaagagaaagaattctttaaaaaaaacaaatttttaagtcttttgagtattctattgggttgggtttgggtctgtcaaagtttttaagattaaagctctgagctttttattcacatacaccaaaaaagagtgtgtcttggtttcttttgggtgtgtttcttttagcaaatgccttaaaaatgcacaagtgaaaccagttgggttgtagtttgagctttgacacataaaaaggcttgagctttagctttgtctgttgtgttgtttagagttttgggttatggcgggtctgatcgatctgaacagcacgacggaggaggaggaggagacgccgtcatctgggtcgtcgtccaattcgtctggctcaaatggtttgatttctgggtctgtttgcttggagctgtggcacgcctgtgctgggccactgatttctttgcccaagaaaggtagtgtggtggtttatcttccacaagggcacttggagcaagtgagtgattttccagcctcggtttatgatctccctgctcatctgttttgccgagttctggatgttaagcttcatgcggagagtggtagtgatgaagtgtacgcacaggttcagttggttcctgaaagtgaggaatttgagcacaaactaggggaaagagaaactgttgcagatggggacgaggatgctgagggttcagagaaatcaactacaccccatatgttctgcaaaacccttactgcttctgatactagcactcatgggggcttctctgtccctcgccgtgctgctgaggattgttttcctcccctggattacagtcaacaaaggccttcacaggagctagtggcaaaggatctgcatggcctggaatggaggttcagacatatctatagggggcagccacgcaggcatttgcttaccactggatggagtgcctttgtgaacaagaagaagctcgtttctggagatgctgtgttgtttctcaggggtgaggatggagaactgagacttggagttagaagggcagcccaagtaaaagcttctgccacttatccaactcctggtagccagcatttaaactataactctgtcacagagctggtggatgctatatctacgaagactgcttttaacgcctattacaatccaagagccagctcatcagaatttataatacctttccgtaagtttttgaggagccttggtcattccttctgtgctggaatgagatttaaaatgcgctttgaaacagaagacgccgcagagcaaagatacactggactggtaacggggattagtgagttggatcccctaagatggcctggttccaagtggaaatgtgtagctgtacggtgggatgatatagatactagcaagcagcatggccgggtttccccatgggaaattgagccatctggttctatttctaattccagtggcttaatggcatctggtctgaagaggtccaggatgggcttatctgcagaaaagcaagaatttccagttcctcatgggattggagcctcagactttggggaatctttaagattccagaaggtcttgcaaggtcaagaagtttcgggttttgatactccttttggttctatagggggtcaaaatcagcatccctctgaatcgaggagagtctttcacggctctattggttctagaggtaatgatctcagaaactcatttgtgaattctgagattgcctcaaaaggctttggtgaatctttccgattccagaaggtcttgcaaggtcaagaaatatttccaagcacaccatacggaagagctccagctactaatgaggctcgtgaatatggttgccctggaatctttgatggttttcaggtgccaagctttagaaatggatggtctacgatgatgcagggcagtaatacacctatgcaccgagctgcccctgtacaggtgtcatcaccatcatctgtgctgatgttccagcaagcaataaatgcaggagccgagttcaattcagtatacaatggtcataaccaacaggaacagagaataatgcaacgcactcattctgaatcagatggtgggaagcaaacatcagcctcgttctgtgaacgaagcttcaccagggagggtcatggtggcatgaattcttttgatcaacatggtatttcacatcctcctcttttgagtcagtcttcattgagaggcagtcaagatatggtttcatcatgcaaaagtagctgcagactgtttggtttctcactgtctgaggaaacacatgccccaaataaagtggacaactccacctcagttacatctgcattagagtctggagcttctatgttccccaatgttgaaccacggtttcattcaaagccgccttcgatgtctgcagctgttgggattccttgtaccaaagaatgggcatttaactggcgtggagaaaggatggaaagttgtttacaaggatagtgacaacgacacagagcttgttgtgacgttccacccagaaatgctaccacaatattatgtaagaaacactaggctagaagatgtagtctttgcgcccgaggattttcgcaggttatgcgtgtgttgtattttatgtaactgaactacatttgaaggtaaaaaaaaagaaaaaaagaagaaggtttgattaagcgcttctgggtgacttgattgtattatgatgaattaagctgtaagaaacggtttgcagaatctatgattgcctcttgaaaaaggggcctatccgaaactgaacaaattgtaccgatttgcaattgttaaataatgttattacttatcgtcccta

SEQ ID NO: 22 - DNA, 2215 bp, Prunus persica
atggggggtctaatcgatctgaacagtgcaacggaggacgaggaaacgccgtcgtctggttcgtcttcaacttcctctgcttctgacgcttcggcttcggcttcggcttcggtgtgcttggagctgtggcacgcgtgtgcgggcccactgatttcgctgccaaagaaagggagtgtggtagtgtatcttccacagggccacttggagcaagtctctgattttccagcttcggcttataatctcccacctcaccttttctgtcgcgttgttgatgtcaagctccatgctgagactggtaccgacgatgtgtatgcgcaggtttcacttgttcctgaaagtgaggaaattgaacacaaactgcgggaaggggaaactgatgcatatggtgaggaggaggatgtcgaagcaattgggaagtcaaccacaccccatatgttctgcaaaacccttactgcttctgatactagcactcatggaggcttctccgtccctcgtcgtgctgctgaggattgttttcctcccctggattacaatcaacaaaggccttcacaagaactcgtagcaaaggatctgcatggcctggagtggaggttcagacatatttatagggggcagccacgaaggcatttgctcaccactggatggagtgcatttgtgaacaagaagaagctcgtctctggagatgcagtgctgtttctcaggggtgatgatggagaactgaggctaggaattagaagggcagcccaggttaaagggtccgctacttatccaactctttgtagccagcaattaaactataacactatcacggacgtggtgaatgctatatccatgaagaatgcatttaacatcttctacaatccaagagccagctcatcagaattcataataccttcccgtaaatttttgaggtcccttgatcattccttttcacctggaatgcggttcaaaatgcgttttgaaacagaagatgcagcagagcgaagatacactgggctgataactggaattagtgaattggatcctgtaagatggcctggttcaaaatggagatgtctagttgtaaggtgggatgatatagacacaagtaagcatggcagggtttccccatgggaaatcgagccatctggttctgtttcaagttcccatagcttaatggcagctggtttgaagagggccaggagtggcttgtctgcagcaaaaacagaatttccagttcctaatgggattggagcatcagactttggggaatctttaaggttccagaaggtcttgcaaggtcaagaaattttaggttttgatactcattttggtggtttaggtggtcagaatcaacatccatctgaaccaaggaggggttttcatggttctagtggttctgggattgctgctggaggtaatggtctcagaaagtcacttgcgcactctgagattacctcaaccggcataggctttggtgaatcattccgattccataaggtcttgcaaggtcaagaaatatttccaagcccaccatatggaagagcttccactaataacgaggctcatgaatatggtggccctggaatttatgatggttttcaggtgccaagctttagaaatgggtggcctgccatgatgcagagcaataatgcacacgtgcgcccatctgcctcgtctgtgcaagtttcatcaccatcgtctgtgttaatgttccagcaagcaatgaatccaggcccggaattcaattcagtatacaatggtcataaccaggaggaacagagagttataaaacggactccatatgtctctgaatcagatggcggaaagcaagcatcatcctcattttgtgaacgtagcttcagcagggaagatcatggaggcatgaattcttacaatcaacatggtatctcaaatcatcctgtaataagtcaatcaacatttagtggcagtcaggatgcggtttcaccatacaaaggcagctgtagactctttggtttctcattgtctgaggaaaaacgtgtcccagacagagagagcaactccacctcaactgcatctacattaaatcctggagtgcagtttcattcaaagcctgcattgatgacatcagcagttggaattacctgtaccaaagaatgggcttttgactggcgtggagaaaggatggaaagctgtttacaaggatagcgatgatacaatggcttgttgcagaagatcaaaggcagggtcttaa

SEQ ID NO: 23 - DNA, 669 bp, Pyrus communis
attgcctcaaaaggcataggctttggtgaatcactccgattccataaggtcttgcaaggtcaagaaatatttccaagctcaccatatggaagagctcccacttctaacaaagctcatgaatatggtggacctggagtctatgatggttttcaggtgcccggctttagaaatggatggtccaccatgatgcagagcaataatacacatgtgcacccatctgccacatctgtgcaagtttcatcaccatcgtctgtgttaatgttccagcaagcaatcaacccagttatggaattcaattcggtatacaatggtcataaccaagaggaacatacagttataaatcgaactccatatgtctctgaatatgacggtggaaggcaaacatcatcctcatttggtgaacgtaacttcagcagggaagataatggtggcacgcattcttacagtatttcaaacgatccagttataagtcgatcaacatttagtggcagtcaggattcagtttcaccaaccaaaggtagctgtagactctttggtttctcattgtctgaggacaaatgtgtcccggatcaagcccctactgctggagtgcggtttcattcaaagcctcctttgatgacttcagcagttggaattacctgtactaaagtaagcaacctctttgctgca

SEQ ID NO: 24 - DNA, 3045 bp, Populus tremula
atggaaaggaagaagcacttgaaaaagaaaagataagagagacagatatagttcccattaatatctctttttctgtctctctctctaacactactgccacacatcgcatccttgcagggtcttcacagcatggcagcattgcggcaggcactgcatctcagttttgcagatcatgagcaaggaaagaaacccatgaaaaattgagaagaaaataaataaaaagttgaaagctttaatttaatttaatttaatactagtaccctttaaagcctttgatttgatatcttaaaaaagcagagagagacaaagggtctctctttttaagagtcttgactctaatctccttttaggcaattgccaaagttgcactataatgcagtcatgaaatctctcctcgctcacaaaagcacttgtcttttaataaaccttcattattgttatcaacagttactccttgttattcttcaagaactctacactgttcctgttgttactgcctttgtttaggaaaggctatagagctgatcaaggctaaaaatggtgggtatgatagatctcaacactattgaagaagatgaaactacaccgtcttgtgggtctttatcttctccatcatcatcctctgctgcttctgctttgagtgcttctggctctggttctagtacctcttctgtttgtttggagctttggcatgcttgtgctggcccactaatatctttgccaaagagagggagtgttgttgtgtatttccctcaaggccacttggaacaactccctgatttgcctcttgcagtttatgatctcccttctcatgtcttctgtcgagttgttgatgtcaagctccatgccgaggcagcaagtgatgaggtgtatgcacaggtctccctggttcctgagagtgaggaaattgagcagaagttgagggaggggatatttgagggggatggtgaggaggaggatggtgaagccactgtgaagatgacaacaccccatatgttctgtaagaccctaactgcttctgacactagcactcatggaggcttttcagtccctcgtcgagctgctgaggactgcttccctcctctggattatactcaacaaaggccttcacaagagcttgtggcaaaggatcttcatggctctgagtggaagtttcgacatatctacaggggtcagccacggaggcatttgctcactactggatggagtgcgtttgtcaataagaaaaaacttgtctctggggatgccgttctctttctcaggggtgaggatggggaattgagactgggagttcgaagagcagcacaagttaaatgtggccctacatttccagctcaatggaatcatcagctgaatcagatctctcctggggatgtagctaatgctatttctactagaagttttttccacatttactacaatccaagggccagctcatcagagttcataataccttttaataaattcttgaagagccttgatcaatccttctcttctggaatgagattcaaaatgcgttttgaaacagaagatgcagcagagagaagatacactggaataataactggagtcagtgagctagatcctgctagatggcctggttcaaaatggaaatgcctgttggtaaggtgggatgatatggaggctaacaggctcagcagggtttctccttgggaagttgagccttctggttctggttctttttccagttccaataactttacggcacctggtttgaagaggagcaggtctggattgccttcatcaaaggcagaatttccaattcctgatgggataggagcaccagactttagggaatcttcaaggtcccaggaggtcttgcaaggtcaagaaattatgagttttaatgctctttatgatggtgttgatggtcagaaccagcacccatctgaaataaggagttgttttcctggttaccacagttctgggattgctgcattaggaagtggtatcagagactcgattgccacttcaaataactcctacaagggcataggctttaacgaatcttatagattccataaggtcttccaaggtcaagaaatttttccaagctcaccatatggaagaatcccaaatgctaatgaggctcgtgaaaattgtagtcttggattctctgatggtgtccaaaggtcaagctcaagctcaagaaatggatggtctacattgatgcagggctataatactcaaattcgacctcctgcacaagtatcatcaccatcttcggtgttaatgtttcagcatgctagcaatccagttccaaagccatcttccaattttaatttcaatgatcatgtgcagcagacagctaccacccgaagttggttttgtggtcctgaaatgcaggggggggatttcaagttgcctgcacattctgagcccagtgtaaaaagaggcggccagtggagcaatagtccttttggtctgtcccatgagcatcttcaacatggtgtttcacaacctattgtagctcaatcagcctttaggggtagtcaagatttggtgtcgtgcaaaagcagctgcagactctttggtttctcattgactgaggataaatgccttgttaataaggaggacaatatgaccttaataacatctccattgaatcctggatcctcctttctgcctcgcgcaggagagcacttccatccaaagcctccagcaataaataatgcagttgggagcagttgtaccgaagcaattctgcaaacccgtgctgaaaattatcgaatatactaatgaggctcgcacaagggatgcttcctgttgcttggttttatatgtattagcttgtgagagaatataattattctcctaaggtaacttggctatatcctaactcctttgactatgcaacagagctgtttgtacctggtactaatctctgttagatttcccatgataacccacattcaagaatgttctcttcatacagtgcacaatccaatctggaaatgtagttgtaatagcgccagatattttatatggttgtcatctctcaatatgttttgttctatgctagcc

SEQ ID NO: 25 - DNA, 2790 bp, Vitis vinifera
atggtggctatgatcgatctcaacaccgtcgacgacgacgagacaccctcgtctgggtcgtcgtcttcctcctcctcatccgcctctgcttctgcttccacagtttgtggttctttgttgtcggcggcgtcgtcggtatgtttggagctgtggcacgcgtgtgctggcccgctcatatcgcttccgaagaaaggcagccttgtggtgtactttccacagggccacctggagcagctttctgattatccggccgtagcctatgatctcccgcctcacgtcttctgtcgagtggttgatgtcaagctccatgccgaggtagttacggatgaagtttacgcacaggtctcgctggttcctgaaaccaagcagattaagcagaaactgcaggaaggggaaattgaagcagatggtggtgaagaagaggatattgagggttctatcaagtccatgacaccccacatgttctgcaaaactcttactgcttcagatactagcacccatgggggtttttctgtcccccgccgagctgcagaggactgttttcctcccctggattacaaacagcagagaccttcacaagagcttgtggccaaagatttgcatggcttcgaatggagattccggcatatctacagggggcagccaaggcggcatttgcttactactggttggagtgcatttgtaaacaagaagaagcttgtgtctggagatgctgtactctttcttaggggtggggatggagaactaagactgggaatccgaagagcagctcaaattaaaggttcgtctcctttcccagctctttgtagccaacagttgaatctcaacacccttacagctgtggtcaatgctatatccacaagaagtgttttcaacatatgctacaatccgagggctagctcatcagagttcataataccgctccgtaaattctcaaagagcattgatcattcattttctgctgggatgaggttcaaaatgcgtgttgaaacagaagatgcagcagaacgaagatatactggactgataactgggatcagtgacatggatcctgttagatggcctggttctaaatggaggtgcctattggtaaggtgggacgatatagaggctaatcgacataacagggtttctccatgggaaattgagctatctggttcgctttctggttctggcagcttgacagttcctggctcaaagaggaccaggattggtttgccgggaactagaccagatttttcagttcccaatgggatgggagtgtcagactttggggaatcttcaaggttccagaaggtcttgcaaggtcaagaaatttttggttttaacactccttatgatggtgttgatacccaggatcatcatccatctgaaataaggtgttttcctggttcaagttgttctgggattgctgcaataggaaatggtgttagaaaccctcttgggaattctgatatttcctataaaggcataggctttggtgaatcttttcgattccataaggtcttgcaaggtcaagaaacatttccaagcccaccatgtggaagagctctgtctgctaaccaggctcatgaaaatggtagctttggaatctttgatggtgttcaagtgccgacttctagaaatggatggcctgcccttgtgcagggatataatgcccacactcacctgtccacaccatcagtgcaagtgtcgtcaccatcatcggtgttaatgttccagcaagcaagcactgctgctcctaacatttactcaatgcatagcgccaataatcaggagaaggagcaagaaattagtaaccggagttcatttgatattcctgaagtgtatggtgaaaagctcacaccatcacgttgtgagcttagtgtcaggggaggaggtcagggaggtatgaatttctttggtctgttaaacgagcataatcaactagctgttccacatcctcttgtaactcaatcagcatttagaggcagtcaagatttagttcctacatgtaaaagtagctgcaggctctttggcttttccttaacggaggaaagaagcattggaaataaagtggacaaccccactcctgttacatcttcattgattcctggaacctcttttctgccccagcagttgcactcagagcctccggtgatgaccaaggcaattggaagcaattgtaccaaagtaagtgacttctatgctgtaagggatatgctttttgatattgcgctgtagcgtactgctgttgtaagatcaaaattgcaatttcacaagctggggagtgttgtagaccaggcaattaatcgctggaagcttgataggcatgatgatttgatttgtgcattgaagcatttatttgatatggagggagggcttctgcatggtgagggaaagttgtttaccaggatcatgaggatgttgtgatgcttgttcgagatgactcatggcaggaaatctgcagcatttgatgaaaaattatgatatttactaatgaagacgtagtgatggcaccaaacatagatgcttatagttgctgagaggcacacatggcatcattgatatgtttttagctcttgggcgaaagaactgtaattattgccataacagtaatgtatcttaacctcccttgctatggagaacaatttaaactaatttactaggttccttggaatactcagttaagaaattacttttaaaactgtatcaaaatattactctatgttgttcatcagttgtgttactgtattgcagctattgcttctgtatctctgcttaacattgttggcttaaggctgtttccca

SEQ ID NO: 26 - DNA, 656 bp, Malus domestica
aacaatgcgcggctgccgttgacgttagagtctacgctcctctctctcctctctctcctctctctctctctctaccgtttataaatcccgtcctcaaacgccacttctacatcaccgcccctccctctgaaatcctctccctctctacgctcctctctctcctctctcttctctctcttctctctctctaccgtttataaatcccctgtcctcaaacgccacttctacatcaccacccccccctctgaaaatcctctttctctctctctctctctctctctctctgtgaaaaagctctctctctctctctctgtgaaaaagttaaactttaattgcaatatgcaatcacaaactatcccatatggaacatggattccgggcacccgagccggccacgcgacgccgtcctcacgcgacgcctcacgtgagcaacacctagcggcggccagcgtacaaaaaatggtgtcggagaatgctgtcacggttgtcggacgacgtggctgctgcatgtgccacgtcgtcaagcggctgctcctcggtcacggggtcaaccctacggttttcggcgatgagccagatctgaaacaagggcgaattctgcagatatccatcacactggcggccgctcgagcatgcatctagagggcccaattcgc

SEQ ID NO: 27 - DNA, 421 bp, Malus domestica
actctcgctcccggagctcctcaaccagtcggagcagctccgtcacgtccggcggcttaggctgcacctgcgcggaggtgcgtgggaagtatacaccaaaggagcgcgagaacaccgcccccttctggggtgtcttcccagagctcaacgaaggcgacggagactttgaaggagtttccggtttgggattcgccggcgatttctgtagccccattgccaccctcaccttcccagcaaccattgcaaaaccccctctccctttcactcaacaccctgtttctctcactctctctctctctctctctctctctctctctctctctctctctctctctctctctctaaaagtgtgatgttcctctctcaaggatttggggtgtgtgattagcttgcataatccagcacagagtgaaggggttac

SEQ ID NO: 28 - protein, 707 aa, Malus domestica
MAGLIDLNSATEDEETPSSGSPSSASSVSDALGSSASVCMELWHACAGPLISLPKKGSVVVYLPQGHLEQVSDFPTSAYDLPPHLFCRVVDVKLHAETGTDDVFAQVSLVPESEEIEHRLREGVTDADAEEDVEAMGTSTTPHMFCKTLTASDTSTHGGFSVPRRAAEDCFPPLDYTQQRPSQELVAKDLHGLEWRFRHIYRGQPRRHLLTTGWSAFVNKKKLVSGDAVLFLRGDDGELRLGIRRAAQFKSSATCPTLCSQQLNYSTITDVVNAIFAKNAFNVYYNPRSSSSEFIIPSHKFLRSLDHCFCAGMRIKMRFETEDAAERRYTGLITGISELDPVRWPGSKWRCLVVRWDDIDTSKHGRVSPWEVERSGSVSSSHTLMTTGLKRSRIGLSATKPEFPVPSMSCNGIGTSDFGESLRFQKVLQGQEISGFDTPFSGLGGLNSHPSEARRVFHGSGGSGIAAGGNGLRQSLVDSEIASKGIGFGESFRFHKVLQGQEIFPSSPYGRAPASNEAHEYGGPGLYDGFQVPGFRNGWSTMMQSNNTNVHSSAPSVQVSSPSSVLMFQQAMNPVAEFNSVYNGHNQEDHRVNRTPHVLEHDGGRQTSSSFGERNFSREDRGGTHSYNQHGISPHPVISQSTISGSQDSVSPIKGSCRLFGFSLSEDKCVPDQEGNPNVGVQFHSKPPLMTSTVGITCTKVSNLFAA

SEQ ID NO: 29 - protein, 707 aa, Malus domestica
MAGLIDLNSATEDEETPSSGSPSSASSVSDALGSSASVCMELWHACAGPLISLPKKGSVVVYLPQGHLEQVLDFPTSAYDLPPHLFCRVVDVKLHAETGTDDVFAQVSLVPESEEIEHRLREGVTDADAEEDVEAMGTSTTPHMFCKTLTASDTSTHGGFSVPRRAAEDCFPPLDYTQQRPSQELVAKDLHGLEWRFRHIYRGQPRRHLLTTGWSAFVNKKKLVSGDAVLFLRGDDGELRLGIRRAAQFKSSATCPTLCSQQLNYSTITDVVNAIFAKNAFNVYYNPRSSSSEFIIPSHKFLRSLDHCFCAGMRIKMRFETEDAAERRYTGLITGISELDPVRWPGSKWRCLVVRWDDIDTSKHGRVSPWEVERSGSVSSSHTLMTTGLKRSRIGLSATKPEFPVPSMSCNGIGTSDFGESLRFQKVLQGQEISGFDTPFSGLGGLNSHPSEARRVFHGSGGSGIAAGGNGLRQSLVDSEIASKGIGFGESFRFHKVLQGQEIFPSSPYGRAPASNEAHEYGGPGLYDGFQVPGFRNGWSTMMQSNNTNVHSSAPSVQVSSPSSVLMFQQAMNPVAEFNSVYNGHNQEDHRVNRTPHVLEHDGGRQTSSSFGERNFSREDRGGTHSYNQHGISPHPVISQSTISGSQDSVSPIKGSCRLFGFSLSEDKCVPDQEGNPNVGVQFHSKPPLMTSTVGITCTKVSNLFAA